European Patent Specification EP 3 955 925 B1, published February 11, 2026. Title: Humanized Anti-PD-L1 Antibodies. Applicant: QLSF Biotherapeutics Inc. Chen , Shihao. Application Unknown. The sequence listing filed with the application follows.

SEQUENCE LISTING (118 sequences)

SEQ ID NO: 1 - protein, 108 aa, Mus musculus
DIQMTQSPASLSVSVGETVTITCRASENIHSNLAWYQQKQGKSPQLLVYGATNLADGVPSRFSGSGSGAQYSLKINSLQSEDFGSYYCQHFWGTPPYAFGGGTKLETK

SEQ ID NO: 2 - protein, 106 aa, Mus musculus
QIVLTQSPAIMSASPGEKVTISCSASSSVFDMYWYQQKPGSSPKPWIYRTSNLASGVPARFSGSGSGTSYFLTISSMEAEDAATYYCQQYQSFPLTFGAGTKLELK

SEQ ID NO: 3 - protein, 107 aa, Mus musculus
DIQMTQSPSSLSASLGERVSLICRASQEISGYLSWLQQKSDGTIKRLIFAASTLDPGVPKRFSGSRSGADYSLTISSLESEDFADYYCLQYAIYPPTFGSGTKLEIK

SEQ ID NO: 4 - protein, 106 aa, Mus musculus
QIVLTQSPAIMSASPGEKVTMTCSASSSVSFMHWYQQKSGTSPKKWIYDTSKLASGVPVRFSGSGSGTSYSLTIINMEAEDAATYYCQQWTYYPPTFGGGTKLEIK

SEQ ID NO: 5 - protein, 107 aa, Mus musculus
DIQMTQSPSSLSASLGERVSLTCRASQEISVYLSWLQQKPDGTIKRLIYAASTLDSGVPQRFRGSRSGSDYSLTISSLESEDFADYYCVQYTSHPYTFGGGTKLEIK

SEQ ID NO: 6 - protein, 108 aa, Mus musculus
DIQMTQSPASLSVSVGETVTITCRASENIHSNLAWYQQKQGKSPQLLVYGATNLADGVPSRFSGSGSGAQYSLKINSLQSEDFGSYYCQHFWGTPPYVFGGGTKLETK

SEQ ID NO: 7 - protein, 115 aa, Mus musculus
QVQLQQPGSELVRPGTSVKLSCKASGYTFTTFWMHWVKQRPGQGLEWIGNIYPGSGTINYDEKFRSKATLTVDTSSNTAYMQVSSLTSEDSAVYYCTTGWDGEHWGQGTTLTVSS

SEQ ID NO: 8 - protein, 121 aa, Mus musculus
EVQLVESGGGLVKPGGSLKLSCAASGFTFSDYGMHWIRQAPEKGLEWIAYIGTTSSIIYYADTVKGRFTISRDNAKNTLFLQMTSLRSEDTAMYYCARRDYGNYYWYLDVWGTGTTVTVSS

SEQ ID NO: 9 - protein, 115 aa, Mus musculus
EVQLQQSGAELVKPGASVKLSCTASGFNIKDTYMHWVQQRPEQGLEWIGRIDPMNGNSKYDPKFQDKATITADTSSNTAYLQLSSLTSEDTAVYYCTSSKWGDYWGQGTTLTVSS

SEQ ID NO: 10 - protein, 121 aa, Mus musculus
EVQLQQSGAELVRPGALVKVSCKASGFNIKDYYIHWVKQRPEQGLEWIGWIDPDNGNTKYDPNFQGKASMTADTSSNTVNLQLSSLTSKDTAVYYCARYGGYGGFYTMDYWGQGTSVTVSS

SEQ ID NO: 11 - protein, 119 aa, Mus musculus
QVQLQQPGTELVKPGASVKLSCKASGYTFTIYWMHWVKQRPGRGLEWIGRIDPNSGDTKYTEKFKNRATLTVDKSSNTAYMQFSSLASDDSAVYYCARGGPNWDGFAYWGQGTLVTVSA

SEQ ID NO: 12 - protein, 115 aa, Mus musculus
QVQLQQPRSELVRPGASVKLSCKASGYTFTTFWMHWVKQRPGQGLEWIGNIYPGSGISNYDEKFKNKATLTVDTSSSTAYMQVSSLTSEDSAVYYCTTGWDGEHWGQGTTLTVSS

SEQ ID NO: 13 - protein, 11 aa, Mus musculus
RASENIHSNLA

SEQ ID NO: 14 - protein, 10 aa, Mus musculus
SASSSVFDMY

SEQ ID NO: 15 - protein, 11 aa, Mus musculus
RASQEISGYLS

SEQ ID NO: 16 - protein, 10 aa, Mus musculus
SASSSVSFMH

SEQ ID NO: 17 - protein, 11 aa, Mus musculus
RASQEISVYLS

SEQ ID NO: 18 - protein, 11 aa, Mus musculus
RASENIHSNLA

SEQ ID NO: 19 - protein, 7 aa, Mus musculus
GATNLAD

SEQ ID NO: 20 - protein, 7 aa, Mus musculus
RTSNLAS

SEQ ID NO: 21 - protein, 7 aa, Mus musculus
AASTLDP

SEQ ID NO: 22 - protein, 7 aa, Mus musculus
DTSKLAS

SEQ ID NO: 23 - protein, 7 aa, Mus musculus
AASTLDS

SEQ ID NO: 24 - protein, 7 aa, Mus musculus
GATNLAD

SEQ ID NO: 25 - protein, 10 aa, Mus musculus
QHFWGTPPYA

SEQ ID NO: 26 - protein, 9 aa, Mus musculus
QQYQSFPLT

SEQ ID NO: 27 - protein, 9 aa, Mus musculus
LQYAIYPPT

SEQ ID NO: 28 - protein, 9 aa, Mus musculus
QQWTYYPPT

SEQ ID NO: 29 - protein, 9 aa, Mus musculus
VQYTSHPYT

SEQ ID NO: 30 - protein, 10 aa, Mus musculus
QHFWGTPPYV

SEQ ID NO: 31 - protein, 5 aa, Mus musculus
TFWMH

SEQ ID NO: 32 - protein, 5 aa, Mus musculus
DYGMH

SEQ ID NO: 33 - protein, 5 aa, Mus musculus
DTYMH

SEQ ID NO: 34 - protein, 5 aa, Mus musculus
DYYIH

SEQ ID NO: 35 - protein, 5 aa, Mus musculus
IYWMH

SEQ ID NO: 36 - protein, 5 aa, Mus musculus
TFWMH

SEQ ID NO: 37 - protein, 17 aa, Mus musculus
NIYPGSGTINYDEKFRS

SEQ ID NO: 38 - protein, 17 aa, Mus musculus
YIGTTSSIIYYADTVKG

SEQ ID NO: 39 - protein, 17 aa, Mus musculus
RIDPMNGNSKYDPKFQD

SEQ ID NO: 40 - protein, 17 aa, Mus musculus
WIDPDNGNTKYDPNFQG

SEQ ID NO: 41 - protein, 17 aa, Mus musculus
RIDPNSGDTKYTEKFKN

SEQ ID NO: 42 - protein, 17 aa, Mus musculus
NIYPGSGISNYDEKFKN

SEQ ID NO: 43 - protein, 6 aa, Mus musculus
GWDGEH

SEQ ID NO: 44 - protein, 12 aa, Mus musculus
RDYGNYYWYLDV

SEQ ID NO: 45 - protein, 6 aa, Mus musculus
SKWGDY

SEQ ID NO: 46 - protein, 12 aa, Mus musculus
YGGYGGFYTMDY

SEQ ID NO: 47 - protein, 10 aa, Mus musculus
GGPNWDGFAY

SEQ ID NO: 48 - protein, 6 aa, Mus musculus
GWDGEH

SEQ ID NO: 49 - protein, 108 aa, Artificial Sequence
  Humanized light chain variable domain
DIQMTQSPSSLSASVGDRVTITCRASENIHSNLAWYQQKPGKAPKLLVYGATNLADGVPSRFSGSGSGAQYTLTISSLQPEDFATYYCQHFWGTPPYAFGGGTKLEIK

SEQ ID NO: 50 - protein, 108 aa, Artificial Sequence
  Humanized light chain variable domain
DIQMTQSPSSLSASVGDRVTITCRASENIHSNLAWYQQKPGKAPQLLVYGATNLADGVPSRFSGSGSGAQYTLTISSLQPEDFATYYCQHFWGTPPYAFGGGTKLEIK

SEQ ID NO: 51 - protein, 108 aa, Artificial Sequence
  Humanized light chain variable domain
DIQMTQSPSSLSVSVGDRVTITCRASENIHSNLAWYQQKPGKAPQLLVYGATNLADGVPSRFSGSGSGAQYTLTISSLQPEDFATYYCQHFWGTPPYAFGGGTKLEIK

SEQ ID NO: 52 - protein, 108 aa, Artificial Sequence
  Humanized light chain variable domain
DIQMTQSPSSLSASVGDRVTITCRASENIHSNLAWYQQKPGKAPKLLVYGATNLADGVPSRFSGSGSGAQYTLTISSLQPEDFATYYCQHFWGTPPYVFGGGTKLEIK

SEQ ID NO: 53 - protein, 108 aa, Artificial Sequence
  Humanized light chain variable domain
DIQMTQSPSSLSASVGDRVTITCRASENIHSNLAWYQQKPGKAPQLLVYGATNLADGVPSRFSGSGSGAQYTLTISSLQPEDFATYYCQHFWGTPPYVFGGGTKLEIK

SEQ ID NO: 54 - protein, 108 aa, Artificial Sequence
  Humanized light chain variable domain
DIQMTQSPSSLSVSVGDRVTITCRASENIHSNLAWYQQKPGKAPQLLVYGATNLADGVPSRFSGSGSGAQYTLTISSLQPEDFATYYCQHFWGTPPYVFGGGTKLEIK

SEQ ID NO: 55 - protein, 106 aa, Artificial Sequence
  Humanized light chain variable domain
EIVLTQSPATLSLSPGERATLSCSASSSVFDMYWYQQKPGQSPRPWIYRTSNLASGIPARFSGSGSGTDFFLTISSLEPEDFAVYYCQQYQSFPLTFGQGTKLELK

SEQ ID NO: 56 - protein, 106 aa, Artificial Sequence
  Humanized light chain variable domain
EIVLTQSPATLSLSPGERVTLSCSASSSVFDMYWYQQKPGQSPRPWIYRTSNLASGIPARFSGSGSGTDFFLTISSLEPEDAAVYYCQQYQSFPLTFGQGTKLELK

SEQ ID NO: 57 - protein, 106 aa, Artificial Sequence
  Humanized light chain variable domain
EIVLTQSPATLSLSPGERVTLSCSASSSVFDMYWYQQKPGSSPRPWIYRTSNLASGVPARFSGSGSGTDFFLTISSLEPEDAAVYYCQQYQSFPLTFGQGTKLELK

SEQ ID NO: 58 - protein, 106 aa, Artificial Sequence
  Humanized light chain variable domain
EIVLTQSPATLSLSPGERVTLSCSASSSVFDMYWYQQKPGSSPRPWIYRTSNLASGVPARFSGSGSGTDYFLTISSMEPEDAATYYCQQYQSFPLTFGQGTKLELK

SEQ ID NO: 59 - protein, 107 aa, Artificial Sequence
  Humanized light chain variable domain
DIQMTQSPSSLSASVGDRVTIICRASQEISGYLSWLQQKPDGTIKSLIYAASTLDPGVPSRFSGSRSGADFTLTISSLQPEDFATYYCLQYAIYPPTFGQGTKLEIK

SEQ ID NO: 60 - protein, 107 aa, Artificial Sequence
  Humanized light chain variable domain
DIQMTQSPSSLSASVGDRVTLICRASQEISGYLSWLQQKPDGTIKRLIFAASTLDPGVPSRFSGSRSGADFTLTISSLQPEDFADYYCLQYAIYPPTFGQGTKLEIK

SEQ ID NO: 61 - protein, 107 aa, Artificial Sequence
  Humanized light chain variable domain
DIQMTQSPSSLSASVGDRVTLICRASQEISGYLSWLQQKPDGTIKRLIFAASTLDPGVPSRFSGSRSGADYTLTISSLQPEDFADYYCLQYAIYPPTFGQGTKLEIK

SEQ ID NO: 62 - protein, 106 aa, Artificial Sequence
  Humanized light chain variable domain
EIVLTQSPATLSLSPGERATLSCSASSSVSFMHWYQQKPGLAPRKLIYDTSKLASGIPDRFSGSGSGTSYTLTISRLEPEDFAVYYCQQWTYYPPTFGQGTKVEIK

SEQ ID NO: 63 - protein, 106 aa, Artificial Sequence
  Humanized light chain variable domain
QIVLTQSPATLSLSPGERATLSCSASSSVSFMHWYQQKPGLAPRKWIYDTSKLASGVPDRFSGSGSGTSYTLTISRLEPEDFAVYYCQQWTYYPPTFGQGTKVEIK

SEQ ID NO: 64 - protein, 107 aa, Artificial Sequence
  Humanized light chain variable domain
DIQMTQSPSSLSASVGDRVTITCRASQEISVYLSWLQQKPGKAPKRLIYAASTLDSGVPSRFSGSGSGSDYTLTISSLQPEDFATYYCVQYTSHPYTFGQGTKVEIK

SEQ ID NO: 65 - protein, 115 aa, Artificial Sequence
  Humanized heavy chain variable domain
QVQLVQSGAEVVKPGASVKLSCKASGYTFTTFWMHWVRQAPGQGLEWIGNIYPGSGTINYDEKFRSRVTLTVDTSISTAYMELSRLRSEDTAVYYCTTGWDGEHWGQGTTLTVSS

SEQ ID NO: 66 - protein, 115 aa, Artificial Sequence
  Humanized heavy chain variable domain
QVQLVQSGAEVVKPGASVKLSCKASGYTFTTFWMHWVRQAPGQGLEWIGNIYPGSGTINYDEKFRSRATLTVDTSISTAYMEVSRLRSEDTAVYYCTTGWDGEHWGQGTTLTVSS

SEQ ID NO: 67 - protein, 115 aa, Artificial Sequence
  Humanized heavy chain variable domain
QVQLVQSGAEVVKPGASVKLSCKASGYTFTTFWMHWVKQAPGQGLEWIGNIYPGSGTINYDEKFRSRATLTVDTSISTAYMEVSRLRSEDTAVYYCTTGWDGEHWGQGTTLTVSS

SEQ ID NO: 68 - protein, 121 aa, Artificial Sequence
  Humanized heavy chain variable domain
EVQLVESGGGLVKPGGSLRLSCAASGFTFSDYGMHWIRQAPGKGLEWVSYIGTTSSIIYYADTVKGRFTISRDNAKNSLYLQMNSLRAEDTAVYYCARRDYGNYYWYLDVWGQGTMVTVSS

SEQ ID NO: 69 - protein, 121 aa, Artificial Sequence
  Humanized heavy chain variable domain
EVQLVESGGGLVKPGGSLRLSCAASGFTFSDYGMHWIRQAPGKGLEWIAYIGTTSSIIYYADTVKGRFTISRDNAKNSLYLQMNSLRAEDTAVYYCARRDYGNYYWYLDVWGTGTMVTVSS

SEQ ID NO: 70 - protein, 121 aa, Artificial Sequence
  Humanized heavy chain variable domain
EVQLVESGGGLVKPGGSLRLSCAASGFTFSDYGMHWIRQAPGKGLEWIAYIGTTSSIIYYADTVKGRFTISRDNAKNSLYLQMNSLRAEDTAMYYCARRDYGNYYWYLDVWGTGTMVTVSS

SEQ ID NO: 71 - protein, 115 aa, Artificial Sequence
  Humanized heavy chain variable domain
QVQLVQSGAEVKKPGASVKVSCKASGFNIKDTYMHWVQQAPGQRLEWMGRIDPMNGNSKYDPKFQDRVTITADTSASTAYLELSSLRSEDTAVYYCTSSKWGDYWGQGTLLTVSS

SEQ ID NO: 72 - protein, 115 aa, Artificial Sequence
  Humanized heavy chain variable domain
QVQLVQSGAEVKKPGASVKVSCKASGFNIKDTYMHWVQQAPGQRLEWMGRIDPMNANSKYDPKFQDRVTITADTSASTAYLELSSLRSEDTAVYYCTSSKWGDYWGQGTLLTVSS

SEQ ID NO: 73 - protein, 115 aa, Artificial Sequence
  Humanized heavy chain variable domain
QVQLVQSGAEVKKPGASVKLSCKASGFNIKDTYMHWVQQAPEQRLEWMGRIDPMNANSKYDPKFQDRVTITADTSASTAYLELSSLRSEDTAVYYCTSSKWGDYWGQGTLLTVSS

SEQ ID NO: 74 - protein, 115 aa, Artificial Sequence
  Humanized heavy chain variable domain
QVQLVQSGAEVKKPGASVKLSCKASGFNIKDTYMHWVQQAPEQRLEWIGRIDPMNANSKYDPKFQDRATITADTSANTAYLELSSLRSEDTAVYYCTSSKWGDYWGQGTLLTVSS

SEQ ID NO: 75 - protein, 115 aa, Artificial Sequence
  Humanized heavy chain variable domain
QVQLQQSGAEVKKPGASVKLSCTASGFNIKDTYMHWVQQAPEQRLEWIGRIDPMNGNSKYDPKFQDRATITADTSANTAYLELSSLRSEDTAVYYCTSSKWGDYWGQGTLLTVSS

SEQ ID NO: 76 - protein, 115 aa, Artificial Sequence
  Humanized heavy chain variable domain
QVQLQQSGAEVKKPGASVKLSCTASGFNIKDTYMHWVQQAPEQRLEWIGRIDPMNANSKYDPKFQDRATITADTSANTAYLELSSLRSEDTAVYYCTSSKWGDYWGQGTLLTVSS

SEQ ID NO: 77 - protein, 121 aa, Artificial Sequence
  Humanized heavy chain variable domain
QVQLVQSGAEVKKPGASVKVSCKASGYNIKDYYIHWVRQAPGQGLEWIGWIDPDNGNTKYDPNFQGRVTMTADTSTSTVYMELSSLRSEDTAVYYCARYGGYGGFYTMDYWGQGTLVTVSS

SEQ ID NO: 78 - protein, 121 aa, Artificial Sequence
  Humanized light chain variable domain
QVQLVQSGAEVKKPGASVKVSCKASGFNIKDYYIHWVRQAPGQGLEWIGWIDPDNGNTKYDPNFQGRATMTADTSTSTVYMELSSLRSEDTAVYYCARYGGYGGFYTMDYWGQGTLVTVSS

SEQ ID NO: 79 - protein, 119 aa, Artificial Sequence
  Humanized heavy chain variable domain
QVQLVQSGAEVKKPGASVKVSCKASGYTFTIYWMHWVRQAPGQGLEWIGRIDPNSGDTKYTEKFKNRATLTVDKSTSTAYMELSSLRSEDTAVYYCARGGPNWDGFAYWGQGTLVTVSS

SEQ ID NO: 80 - protein, 119 aa, Artificial Sequence
  Humanized heavy chain variable domain
QVQLVQSGAEVKKPGASVKVSCKASGYTFTIYWMHWVKQRPGQGLEWIGRIDPNSGDTKYTEKFKNRATLTVDKSTSTAYMEFSSLRSEDTAVYYCARGGPNWDGFAYWGQGTLVTVSS

SEQ ID NO: 81 - protein, 115 aa, Artificial Sequence
  Humanized heavy chain variable domain
QVQLVQSGAEVVKPGASVKLSCKASGYTFTTFWMHWVRQAPGQGLEWIGNIYPGSGISNYDEKFKNRVTLTVDTSISTAYMELSRLRSEDTAVYYCTTGWDGEHWGQGTTLTVSS

SEQ ID NO: 82 - protein, 115 aa, Artificial Sequence
  Humanized heavy chain variable domain
QVQLVQSGAEVVKPGASVKLSCKASGYTFTTFWMHWVRQAPGQGLEWIGNIYPGSGISNYDEKFKNRATLTVDTSISTAYMEVSRLRSEDTAVYYCTTGWDGEHWGQGTTLTVSS

SEQ ID NO: 83 - protein, 115 aa, Artificial Sequence
  Humanized heavy chain variable domain
QVQLVQSGAEVVKPGASVKLSCKASGYTFTTFWMHWVKQAPGQGLEWIGNIYPGSGISNYDEKFKNRATLTVDTSISTAYMEVSRLRSEDTAVYYCTTGWDGEHWGQGTTLTVSS

SEQ ID NO: 84 - protein, 215 aa, Artificial Sequence
  Humanized light chains
DIQMTQSPSSLSASVGDRVTITCRASENIHSNLAWYQQKPGKAPKLLVYGATNLADGVPSRFSGSGSGAQYTLTISSLQPEDFATYYCQHFWGTPPYAFGGGTKLEIKRTVAAPSVFIFPPSDEQLKSGTASVVCLLNNFYPREAKVQWKVDNALQSGNSQESVTEQDSKDSTYSLSSTLTLSKADYEKHKVYACEVTHQGLSSPVTKSFNRGEC

SEQ ID NO: 85 - protein, 215 aa, Artificial Sequence
  Humanized light chains
DIQMTQSPSSLSASVGDRVTITCRASENIHSNLAWYQQKPGKAPQLLVYGATNLADGVPSRFSGSGSGAQYTLTISSLQPEDFATYYCQHFWGTPPYAFGGGTKLEIKRTVAAPSVFIFPPSDEQLKSGTASVVCLLNNFYPREAKVQWKVDNALQSGNSQESVTEQDSKDSTYSLSSTLTLSKADYEKHKVYACEVTHQGLSSPVTKSFNRGEC

SEQ ID NO: 86 - protein, 215 aa, Artificial Sequence
  Humanized light chains
DIQMTQSPSSLSVSVGDRVTITCRASENIHSNLAWYQQKPGKAPQLLVYGATNLADGVPSRFSGSGSGAQYTLTISSLQPEDFATYYCQHFWGTPPYAFGGGTKLEIKRTVAAPSVFIFPPSDEQLKSGTASVVCLLNNFYPREAKVQWKVDNALQSGNSQESVTEQDSKDSTYSLSSTLTLSKADYEKHKVYACEVTHQGLSSPVTKSFNRGEC

SEQ ID NO: 87 - protein, 215 aa, Artificial Sequence
  Humanized light chains
DIQMTQSPSSLSASVGDRVTITCRASENIHSNLAWYQQKPGKAPKLLVYGATNLADGVPSRFSGSGSGAQYTLTISSLQPEDFATYYCQHFWGTPPYVFGGGTKLEIKRTVAAPSVFIFPPSDEQLKSGTASVVCLLNNFYPREAKVQWKVDNALQSGNSQESVTEQDSKDSTYSLSSTLTLSKADYEKHKVYACEVTHQGLSSPVTKSFNRGEC

SEQ ID NO: 88 - protein, 215 aa, Artificial Sequence
  Humanized light chains
DIQMTQSPSSLSASVGDRVTITCRASENIHSNLAWYQQKPGKAPQLLVYGATNLADGVPSRFSGSGSGAQYTLTISSLQPEDFATYYCQHFWGTPPYVFGGGTKLEIKRTVAAPSVFIFPPSDEQLKSGTASVVCLLNNFYPREAKVQWKVDNALQSGNSQESVTEQDSKDSTYSLSSTLTLSKADYEKHKVYACEVTHQGLSSPVTKSFNRGEC

SEQ ID NO: 89 - protein, 215 aa, Artificial Sequence
  Humanized light chains
DIQMTQSPSSLSVSVGDRVTITCRASENIHSNLAWYQQKPGKAPQLLVYGATNLADGVPSRFSGSGSGAQYTLTISSLQPEDFATYYCQHFWGTPPYVFGGGTKLEIKRTVAAPSVFIFPPSDEQLKSGTASVVCLLNNFYPREAKVQWKVDNALQSGNSQESVTEQDSKDSTYSLSSTLTLSKADYEKHKVYACEVTHQGLSSPVTKSFNRGEC

SEQ ID NO: 90 - protein, 213 aa, Artificial Sequence
  Humanized light chains
EIVLTQSPATLSLSPGERATLSCSASSSVFDMYWYQQKPGQSPRPWIYRTSNLASGIPARFSGSGSGTDFFLTISSLEPEDFAVYYCQQYQSFPLTFGQGTKLELKRTVAAPSVFIFPPSDEQLKSGTASVVCLLNNFYPREAKVQWKVDNALQSGNSQESVTEQDSKDSTYSLSSTLTLSKADYEKHKVYACEVTHQGLSSPVTKSFNRGEC

SEQ ID NO: 91 - protein, 213 aa, Artificial Sequence
  Humanized light chains
EIVLTQSPATLSLSPGERVTLSCSASSSVFDMYWYQQKPGQSPRPWIYRTSNLASGIPARFSGSGSGTDFFLTISSLEPEDAAVYYCQQYQSFPLTFGQGTKLELKRTVAAPSVFIFPPSDEQLKSGTASVVCLLNNFYPREAKVQWKVDNALQSGNSQESVTEQDSKDSTYSLSSTLTLSKADYEKHKVYACEVTHQGLSSPVTKSFNRGEC

SEQ ID NO: 92 - protein, 213 aa, Artificial Sequence
  Humanized light chains
EIVLTQSPATLSLSPGERVTLSCSASSSVFDMYWYQQKPGSSPRPWIYRTSNLASGVPARFSGSGSGTDFFLTISSLEPEDAAVYYCQQYQSFPLTFGQGTKLELKRTVAAPSVFIFPPSDEQLKSGTASVVCLLNNFYPREAKVQWKVDNALQSGNSQESVTEQDSKDSTYSLSSTLTLSKADYEKHKVYACEVTHQGLSSPVTKSFNRGEC

SEQ ID NO: 93 - protein, 213 aa, Artificial Sequence
  Humanized light chains
EIVLTQSPATLSLSPGERVTLSCSASSSVFDMYWYQQKPGSSPRPWIYRTSNLASGVPARFSGSGSGTDYFLTISSMEPEDAATYYCQQYQSFPLTFGQGTKLELKRTVAAPSVFIFPPSDEQLKSGTASVVCLLNNFYPREAKVQWKVDNALQSGNSQESVTEQDSKDSTYSLSSTLTLSKADYEKHKVYACEVTHQGLSSPVTKSFNRGEC

SEQ ID NO: 94 - protein, 214 aa, Artificial Sequence
  Humanized light chains
DIQMTQSPSSLSASVGDRVTIICRASQEISGYLSWLQQKPDGTIKSLIYAASTLDPGVPSRFSGSRSGADFTLTISSLQPEDFATYYCLQYAIYPPTFGQGTKLEIKRTVAAPSVFIFPPSDEQLKSGTASVVCLLNNFYPREAKVQWKVDNALQSGNSQESVTEQDSKDSTYSLSSTLTLSKADYEKHKVYACEVTHQGLSSPVTKSFNRGEC

SEQ ID NO: 95 - protein, 214 aa, Artificial Sequence
  Humanized light chains
DIQMTQSPSSLSASVGDRVTLICRASQEISGYLSWLQQKPDGTIKRLIFAASTLDPGVPSRFSGSRSGADFTLTISSLQPEDFADYYCLQYAIYPPTFGQGTKLEIKRTVAAPSVFIFPPSDEQLKSGTASVVCLLNNFYPREAKVQWKVDNALQSGNSQESVTEQDSKDSTYSLSSTLTLSKADYEKHKVYACEVTHQGLSSPVTKSFNRGEC

SEQ ID NO: 96 - protein, 214 aa, Artificial Sequence
  Humanized light chains
DIQMTQSPSSLSASVGDRVTLICRASQEISGYLSWLQQKPDGTIKRLIFAASTLDPGVPSRFSGSRSGADYTLTISSLQPEDFADYYCLQYAIYPPTFGQGTKLEIKRTVAAPSVFIFPPSDEQLKSGTASVVCLLNNFYPREAKVQWKVDNALQSGNSQESVTEQDSKDSTYSLSSTLTLSKADYEKHKVYACEVTHQGLSSPVTKSFNRGEC

SEQ ID NO: 97 - protein, 213 aa, Artificial Sequence
  Humanized light chains
EIVLTQSPATLSLSPGERATLSCSASSSVSFMHWYQQKPGLAPRKLIYDTSKLASGIPDRFSGSGSGTSYTLTISRLEPEDFAVYYCQQWTYYPPTFGQGTKVEIKRTVAAPSVFIFPPSDEQLKSGTASVVCLLNNFYPREAKVQWKVDNALQSGNSQESVTEQDSKDSTYSLSSTLTLSKADYEKHKVYACEVTHQGLSSPVTKSFNRGEC

SEQ ID NO: 98 - protein, 213 aa, Artificial Sequence
  Humanized light chains
QIVLTQSPATLSLSPGERATLSCSASSSVSFMHWYQQKPGLAPRKWIYDTSKLASGVPDRFSGSGSGTSYTLTISRLEPEDFAVYYCQQWTYYPPTFGQGTKVEIKRTVAAPSVFIFPPSDEQLKSGTASVVCLLNNFYPREAKVQWKVDNALQSGNSQESVTEQDSKDSTYSLSSTLTLSKADYEKHKVYACEVTHQGLSSPVTKSFNRGEC

SEQ ID NO: 99 - protein, 214 aa, Artificial Sequence
  Humanized light chains
DIQMTQSPSSLSASVGDRVTITCRASQEISVYLSWLQQKPGKAPKRLIYAASTLDSGVPSRFSGSGSGSDYTLTISSLQPEDFATYYCVQYTSHPYTFGQGTKVEIKRTVAAPSVFIFPPSDEQLKSGTASVVCLLNNFYPREAKVQWKVDNALQSGNSQESVTEQDSKDSTYSLSSTLTLSKADYEKHKVYACEVTHQGLSSPVTKSFNRGEC

SEQ ID NO: 100 - protein, 445 aa, Artificial Sequence
  Humanized heavy chains
QVQLVQSGAEVVKPGASVKLSCKASGYTFTTFWMHWVRQAPGQGLEWIGNIYPGSGTINYDEKFRSRVTLTVDTSISTAYMELSRLRSEDTAVYYCTTGWDGEHWGQGTTLTVSSASTKGPSVFPLAPSSKSTSGGTAALGCLVKDYFPEPVTVSWNSGALTSGVHTFPAVLQSSGLYSLSSVVTVPSSSLGTQTYICNVNHKPSNTKVDKKVEPKSCDKTHTCPPCPAPELLGGPSVFLFPPKPKDTLMISRTPEVTCVVVDVSHEDPEVKFNWYVDGVEVHNAKTKPREEQYNSTYRVVSVLTVLHQDWLNGKEYKCKVSNKALPAPIEKTISKAKGQPREPQVYTLPPSRDELTKNQVSLTCLVKGFYPSDIAVEWESNGQPENNYKTTPPVLDSDGSFFLYSKLTVDKSRWQQGNVFSCSVMHEALHNHYTQKSLSLSPGK

SEQ ID NO: 101 - protein, 445 aa, Artificial Sequence
  Humanized heavy chains
QVQLVQSGAEVVKPGASVKLSCKASGYTFTTFWMHWVRQAPGQGLEWIGNIYPGSGTINYDEKFRSRATLTVDTSISTAYMEVSRLRSEDTAVYYCTTGWDGEHWGQGTTLTVSSASTKGPSVFPLAPSSKSTSGGTAALGCLVKDYFPEPVTVSWNSGALTSGVHTFPAVLQSSGLYSLSSVVTVPSSSLGTQTYICNVNHKPSNTKVDKKVEPKSCDKTHTCPPCPAPELLGGPSVFLFPPKPKDTLMISRTPEVTCVVVDVSHEDPEVKFNWYVDGVEVHNAKTKPREEQYNSTYRVVSVLTVLHQDWLNGKEYKCKVSNKALPAPIEKTISKAKGQPREPQVYTLPPSRDELTKNQVSLTCLVKGFYPSDIAVEWESNGQPENNYKTTPPVLDSDGSFFLYSKLTVDKSRWQQGNVFSCSVMHEALHNHYTQKSLSLSPGK

SEQ ID NO: 102 - protein, 445 aa, Artificial Sequence
  Humanized heavy chains
QVQLVQSGAEVVKPGASVKLSCKASGYTFTTFWMHWVKQAPGQGLEWIGNIYPGSGTINYDEKFRSRATLTVDTSISTAYMEVSRLRSEDTAVYYCTTGWDGEHWGQGTTLTVSSASTKGPSVFPLAPSSKSTSGGTAALGCLVKDYFPEPVTVSWNSGALTSGVHTFPAVLQSSGLYSLSSVVTVPSSSLGTQTYICNVNHKPSNTKVDKKVEPKSCDKTHTCPPCPAPELLGGPSVFLFPPKPKDTLMISRTPEVTCVVVDVSHEDPEVKFNWYVDGVEVHNAKTKPREEQYNSTYRVVSVLTVLHQDWLNGKEYKCKVSNKALPAPIEKTISKAKGQPREPQVYTLPPSRDELTKNQVSLTCLVKGFYPSDIAVEWESNGQPENNYKTTPPVLDSDGSFFLYSKLTVDKSRWQQGNVFSCSVMHEALHNHYTQKSLSLSPGK

SEQ ID NO: 103 - protein, 451 aa, Artificial Sequence
  Humanized heavy chains
EVQLVESGGGLVKPGGSLRLSCAASGFTFSDYGMHWIRQAPGKGLEWVSYIGTTSSIIYYADTVKGRFTISRDNAKNSLYLQMNSLRAEDTAVYYCARRDYGNYYWYLDVWGQGTMVTVSSASTKGPSVFPLAPSSKSTSGGTAALGCLVKDYFPEPVTVSWNSGALTSGVHTFPAVLQSSGLYSLSSVVTVPSSSLGTQTYICNVNHKPSNTKVDKKVEPKSCDKTHTCPPCPAPELLGGPSVFLFPPKPKDTLMISRTPEVTCVVVDVSHEDPEVKFNWYVDGVEVHNAKTKPREEQYNSTYRVVSVLTVLHQDWLNGKEYKCKVSNKALPAPIEKTISKAKGQPREPQVYTLPPSRDELTKNQVSLTCLVKGFYPSDIAVEWESNGQPENNYKTTPPVLDSDGSFFLYSKLTVDKSRWQQGNVFSCSVMHEALHNHYTQKSLSLSPGK

SEQ ID NO: 104 - protein, 451 aa, Artificial Sequence
  Humanized heavy chains
EVQLVESGGGLVKPGGSLRLSCAASGFTFSDYGMHWIRQAPGKGLEWIAYIGTTSSIIYYADTVKGRFTISRDNAKNSLYLQMNSLRAEDTAVYYCARRDYGNYYWYLDVWGTGTMVTVSSASTKGPSVFPLAPSSKSTSGGTAALGCLVKDYFPEPVTVSWNSGALTSGVHTFPAVLQSSGLYSLSSVVTVPSSSLGTQTYICNVNHKPSNTKVDKKVEPKSCDKTHTCPPCPAPELLGGPSVFLFPPKPKDTLMISRTPEVTCVVVDVSHEDPEVKFNWYVDGVEVHNAKTKPREEQYNSTYRVVSVLTVLHQDWLNGKEYKCKVSNKALPAPIEKTISKAKGQPREPQVYTLPPSRDELTKNQVSLTCLVKGFYPSDIAVEWESNGQPENNYKTTPPVLDSDGSFFLYSKLTVDKSRWQQGNVFSCSVMHEALHNHYTQKSLSLSPGK

SEQ ID NO: 105 - protein, 451 aa, Artificial Sequence
  Humanized heavy chains
EVQLVESGGGLVKPGGSLRLSCAASGFTFSDYGMHWIRQAPGKGLEWIAYIGTTSSIIYYADTVKGRFTISRDNAKNSLYLQMNSLRAEDTAMYYCARRDYGNYYWYLDVWGTGTMVTVSSASTKGPSVFPLAPSSKSTSGGTAALGCLVKDYFPEPVTVSWNSGALTSGVHTFPAVLQSSGLYSLSSVVTVPSSSLGTQTYICNVNHKPSNTKVDKKVEPKSCDKTHTCPPCPAPELLGGPSVFLFPPKPKDTLMISRTPEVTCVVVDVSHEDPEVKFNWYVDGVEVHNAKTKPREEQYNSTYRVVSVLTVLHQDWLNGKEYKCKVSNKALPAPIEKTISKAKGQPREPQVYTLPPSRDELTKNQVSLTCLVKGFYPSDIAVEWESNGQPENNYKTTPPVLDSDGSFFLYSKLTVDKSRWQQGNVFSCSVMHEALHNHYTQKSLSLSPGK

SEQ ID NO: 106 - protein, 445 aa, Artificial Sequence
  Humanized heavy chains
QVQLVQSGAEVKKPGASVKVSCKASGFNIKDTYMHWVQQAPGQRLEWMGRIDPMNGNSKYDPKFQDRVTITADTSASTAYLELSSLRSEDTAVYYCTSSKWGDYWGQGTLLTVSSASTKGPSVFPLAPSSKSTSGGTAALGCLVKDYFPEPVTVSWNSGALTSGVHTFPAVLQSSGLYSLSSVVTVPSSSLGTQTYICNVNHKPSNTKVDKKVEPKSCDKTHTCPPCPAPELLGGPSVFLFPPKPKDTLMISRTPEVTCVVVDVSHEDPEVKFNWYVDGVEVHNAKTKPREEQYNSTYRVVSVLTVLHQDWLNGKEYKCKVSNKALPAPIEKTISKAKGQPREPQVYTLPPSRDELTKNQVSLTCLVKGFYPSDIAVEWESNGQPENNYKTTPPVLDSDGSFFLYSKLTVDKSRWQQGNVFSCSVMHEALHNHYTQKSLSLSPGK

SEQ ID NO: 107 - protein, 445 aa, Artificial Sequence
  Humanized heavy chains
QVQLVQSGAEVKKPGASVKVSCKASGFNIKDTYMHWVQQAPGQRLEWMGRIDPMNANSKYDPKFQDRVTITADTSASTAYLELSSLRSEDTAVYYCTSSKWGDYWGQGTLLTVSSASTKGPSVFPLAPSSKSTSGGTAALGCLVKDYFPEPVTVSWNSGALTSGVHTFPAVLQSSGLYSLSSVVTVPSSSLGTQTYICNVNHKPSNTKVDKKVEPKSCDKTHTCPPCPAPELLGGPSVFLFPPKPKDTLMISRTPEVTCVVVDVSHEDPEVKFNWYVDGVEVHNAKTKPREEQYNSTYRVVSVLTVLHQDWLNGKEYKCKVSNKALPAPIEKTISKAKGQPREPQVYTLPPSRDELTKNQVSLTCLVKGFYPSDIAVEWESNGQPENNYKTTPPVLDSDGSFFLYSKLTVDKSRWQQGNVFSCSVMHEALHNHYTQKSLSLSPGK

SEQ ID NO: 108 - protein, 445 aa, Artificial Sequence
  Humanized heavy chains
QVQLVQSGAEVKKPGASVKLSCKASGFNIKDTYMHWVQQAPEQRLEWMGRIDPMNANSKYDPKFQDRVTITADTSASTAYLELSSLRSEDTAVYYCTSSKWGDYWGQGTLLTVSSASTKGPSVFPLAPSSKSTSGGTAALGCLVKDYFPEPVTVSWNSGALTSGVHTFPAVLQSSGLYSLSSVVTVPSSSLGTQTYICNVNHKPSNTKVDKKVEPKSCDKTHTCPPCPAPELLGGPSVFLFPPKPKDTLMISRTPEVTCVVVDVSHEDPEVKFNWYVDGVEVHNAKTKPREEQYNSTYRVVSVLTVLHQDWLNGKEYKCKVSNKALPAPIEKTISKAKGQPREPQVYTLPPSRDELTKNQVSLTCLVKGFYPSDIAVEWESNGQPENNYKTTPPVLDSDGSFFLYSKLTVDKSRWQQGNVFSCSVMHEALHNHYTQKSLSLSPGK

SEQ ID NO: 109 - protein, 445 aa, Artificial Sequence
  Humanized heavy chains
QVQLVQSGAEVKKPGASVKLSCKASGFNIKDTYMHWVQQAPEQRLEWIGRIDPMNANSKYDPKFQDRATITADTSANTAYLELSSLRSEDTAVYYCTSSKWGDYWGQGTLLTVSSASTKGPSVFPLAPSSKSTSGGTAALGCLVKDYFPEPVTVSWNSGALTSGVHTFPAVLQSSGLYSLSSVVTVPSSSLGTQTYICNVNHKPSNTKVDKKVEPKSCDKTHTCPPCPAPELLGGPSVFLFPPKPKDTLMISRTPEVTCVVVDVSHEDPEVKFNWYVDGVEVHNAKTKPREEQYNSTYRVVSVLTVLHQDWLNGKEYKCKVSNKALPAPIEKTISKAKGQPREPQVYTLPPSRDELTKNQVSLTCLVKGFYPSDIAVEWESNGQPENNYKTTPPVLDSDGSFFLYSKLTVDKSRWQQGNVFSCSVMHEALHNHYTQKSLSLSPGK

SEQ ID NO: 110 - protein, 445 aa, Artificial Sequence
  Humanized heavy chains
QVQLQQSGAEVKKPGASVKLSCTASGFNIKDTYMHWVQQAPEQRLEWIGRIDPMNGNSKYDPKFQDRATITADTSANTAYLELSSLRSEDTAVYYCTSSKWGDYWGQGTLLTVSSASTKGPSVFPLAPSSKSTSGGTAALGCLVKDYFPEPVTVSWNSGALTSGVHTFPAVLQSSGLYSLSSVVTVPSSSLGTQTYICNVNHKPSNTKVDKKVEPKSCDKTHTCPPCPAPELLGGPSVFLFPPKPKDTLMISRTPEVTCVVVDVSHEDPEVKFNWYVDGVEVHNAKTKPREEQYNSTYRVVSVLTVLHQDWLNGKEYKCKVSNKALPAPIEKTISKAKGQPREPQVYTLPPSRDELTKNQVSLTCLVKGFYPSDIAVEWESNGQPENNYKTTPPVLDSDGSFFLYSKLTVDKSRWQQGNVFSCSVMHEALHNHYTQKSLSLSPGK

SEQ ID NO: 111 - protein, 445 aa, Artificial Sequence
  Humanized heavy chains
QVQLQQSGAEVKKPGASVKLSCTASGFNIKDTYMHWVQQAPEQRLEWIGRIDPMNANSKYDPKFQDRATITADTSANTAYLELSSLRSEDTAVYYCTSSKWGDYWGQGTLLTVSSASTKGPSVFPLAPSSKSTSGGTAALGCLVKDYFPEPVTVSWNSGALTSGVHTFPAVLQSSGLYSLSSVVTVPSSSLGTQTYICNVNHKPSNTKVDKKVEPKSCDKTHTCPPCPAPELLGGPSVFLFPPKPKDTLMISRTPEVTCVVVDVSHEDPEVKFNWYVDGVEVHNAKTKPREEQYNSTYRVVSVLTVLHQDWLNGKEYKCKVSNKALPAPIEKTISKAKGQPREPQVYTLPPSRDELTKNQVSLTCLVKGFYPSDIAVEWESNGQPENNYKTTPPVLDSDGSFFLYSKLTVDKSRWQQGNVFSCSVMHEALHNHYTQKSLSLSPGK

SEQ ID NO: 112 - protein, 451 aa, Artificial Sequence
  Humanized heavy chains
QVQLVQSGAEVKKPGASVKVSCKASGYNIKDYYIHWVRQAPGQGLEWIGWIDPDNGNTKYDPNFQGRVTMTADTSTSTVYMELSSLRSEDTAVYYCARYGGYGGFYTMDYWGQGTLVTVSSASTKGPSVFPLAPSSKSTSGGTAALGCLVKDYFPEPVTVSWNSGALTSGVHTFPAVLQSSGLYSLSSVVTVPSSSLGTQTYICNVNHKPSNTKVDKKVEPKSCDKTHTCPPCPAPELLGGPSVFLFPPKPKDTLMISRTPEVTCVVVDVSHEDPEVKFNWYVDGVEVHNAKTKPREEQYNSTYRVVSVLTVLHQDWLNGKEYKCKVSNKALPAPIEKTISKAKGQPREPQVYTLPPSRDELTKNQVSLTCLVKGFYPSDIAVEWESNGQPENNYKTTPPVLDSDGSFFLYSKLTVDKSRWQQGNVFSCSVMHEALHNHYTQKSLSLSPGK

SEQ ID NO: 113 - protein, 451 aa, Artificial Sequence
  Humanized heavy chains
QVQLVQSGAEVKKPGASVKVSCKASGFNIKDYYIHWVRQAPGQGLEWIGWIDPDNGNTKYDPNFQGRATMTADTSTSTVYMELSSLRSEDTAVYYCARYGGYGGFYTMDYWGQGTLVTVSSASTKGPSVFPLAPSSKSTSGGTAALGCLVKDYFPEPVTVSWNSGALTSGVHTFPAVLQSSGLYSLSSVVTVPSSSLGTQTYICNVNHKPSNTKVDKKVEPKSCDKTHTCPPCPAPELLGGPSVFLFPPKPKDTLMISRTPEVTCVVVDVSHEDPEVKFNWYVDGVEVHNAKTKPREEQYNSTYRVVSVLTVLHQDWLNGKEYKCKVSNKALPAPIEKTISKAKGQPREPQVYTLPPSRDELTKNQVSLTCLVKGFYPSDIAVEWESNGQPENNYKTTPPVLDSDGSFFLYSKLTVDKSRWQQGNVFSCSVMHEALHNHYTQKSLSLSPGK

SEQ ID NO: 114 - protein, 449 aa, Artificial Sequence
  Humanized heavy chains
QVQLVQSGAEVKKPGASVKVSCKASGYTFTIYWMHWVRQAPGQGLEWIGRIDPNSGDTKYTEKFKNRATLTVDKSTSTAYMELSSLRSEDTAVYYCARGGPNWDGFAYWGQGTLVTVSSASTKGPSVFPLAPSSKSTSGGTAALGCLVKDYFPEPVTVSWNSGALTSGVHTFPAVLQSSGLYSLSSVVTVPSSSLGTQTYICNVNHKPSNTKVDKKVEPKSCDKTHTCPPCPAPELLGGPSVFLFPPKPKDTLMISRTPEVTCVVVDVSHEDPEVKFNWYVDGVEVHNAKTKPREEQYNSTYRVVSVLTVLHQDWLNGKEYKCKVSNKALPAPIEKTISKAKGQPREPQVYTLPPSRDELTKNQVSLTCLVKGFYPSDIAVEWESNGQPENNYKTTPPVLDSDGSFFLYSKLTVDKSRWQQGNVFSCSVMHEALHNHYTQKSLSLSPGK

SEQ ID NO: 115 - protein, 449 aa, Artificial Sequence
  Humanized heavy chains
QVQLVQSGAEVKKPGASVKVSCKASGYTFTIYWMHWVKQRPGQGLEWIGRIDPNSGDTKYTEKFKNRATLTVDKSTSTAYMEFSSLRSEDTAVYYCARGGPNWDGFAYWGQGTLVTVSSASTKGPSVFPLAPSSKSTSGGTAALGCLVKDYFPEPVTVSWNSGALTSGVHTFPAVLQSSGLYSLSSVVTVPSSSLGTQTYICNVNHKPSNTKVDKKVEPKSCDKTHTCPPCPAPELLGGPSVFLFPPKPKDTLMISRTPEVTCVVVDVSHEDPEVKFNWYVDGVEVHNAKTKPREEQYNSTYRVVSVLTVLHQDWLNGKEYKCKVSNKALPAPIEKTISKAKGQPREPQVYTLPPSRDELTKNQVSLTCLVKGFYPSDIAVEWESNGQPENNYKTTPPVLDSDGSFFLYSKLTVDKSRWQQGNVFSCSVMHEALHNHYTQKSLSLSPGK

SEQ ID NO: 116 - protein, 445 aa, Artificial Sequence
  Humanized heavy chains
QVQLVQSGAEVVKPGASVKLSCKASGYTFTTFWMHWVRQAPGQGLEWIGNIYPGSGISNYDEKFKNRVTLTVDTSISTAYMELSRLRSEDTAVYYCTTGWDGEHWGQGTTLTVSSASTKGPSVFPLAPSSKSTSGGTAALGCLVKDYFPEPVTVSWNSGALTSGVHTFPAVLQSSGLYSLSSVVTVPSSSLGTQTYICNVNHKPSNTKVDKKVEPKSCDKTHTCPPCPAPELLGGPSVFLFPPKPKDTLMISRTPEVTCVVVDVSHEDPEVKFNWYVDGVEVHNAKTKPREEQYNSTYRVVSVLTVLHQDWLNGKEYKCKVSNKALPAPIEKTISKAKGQPREPQVYTLPPSRDELTKNQVSLTCLVKGFYPSDIAVEWESNGQPENNYKTTPPVLDSDGSFFLYSKLTVDKSRWQQGNVFSCSVMHEALHNHYTQKSLSLSPGK

SEQ ID NO: 117 - protein, 445 aa, Artificial Sequence
  Humanized heavy chains
QVQLVQSGAEVVKPGASVKLSCKASGYTFTTFWMHWVRQAPGQGLEWIGNIYPGSGISNYDEKFKNRATLTVDTSISTAYMEVSRLRSEDTAVYYCTTGWDGEHWGQGTTLTVSSASTKGPSVFPLAPSSKSTSGGTAALGCLVKDYFPEPVTVSWNSGALTSGVHTFPAVLQSSGLYSLSSVVTVPSSSLGTQTYICNVNHKPSNTKVDKKVEPKSCDKTHTCPPCPAPELLGGPSVFLFPPKPKDTLMISRTPEVTCVVVDVSHEDPEVKFNWYVDGVEVHNAKTKPREEQYNSTYRVVSVLTVLHQDWLNGKEYKCKVSNKALPAPIEKTISKAKGQPREPQVYTLPPSRDELTKNQVSLTCLVKGFYPSDIAVEWESNGQPENNYKTTPPVLDSDGSFFLYSKLTVDKSRWQQGNVFSCSVMHEALHNHYTQKSLSLSPGK

SEQ ID NO: 118 - protein, 445 aa, Artificial Sequence
  Humanized heavy chains
QVQLVQSGAEVVKPGASVKLSCKASGYTFTTFWMHWVKQAPGQGLEWIGNIYPGSGISNYDEKFKNRATLTVDTSISTAYMEVSRLRSEDTAVYYCTTGWDGEHWGQGTTLTVSSASTKGPSVFPLAPSSKSTSGGTAALGCLVKDYFPEPVTVSWNSGALTSGVHTFPAVLQSSGLYSLSSVVTVPSSSLGTQTYICNVNHKPSNTKVDKKVEPKSCDKTHTCPPCPAPELLGGPSVFLFPPKPKDTLMISRTPEVTCVVVDVSHEDPEVKFNWYVDGVEVHNAKTKPREEQYNSTYRVVSVLTVLHQDWLNGKEYKCKVSNKALPAPIEKTISKAKGQPREPQVYTLPPSRDELTKNQVSLTCLVKGFYPSDIAVEWESNGQPENNYKTTPPVLDSDGSFFLYSKLTVDKSRWQQGNVFSCSVMHEALHNHYTQKSLSLSPGK